European Patent Specification EP 3 487 985 B1, published November 8, 2023. Title: METHOD FOR PREVENTING OR TREATING MOVEMENT DISORDERS WITH LACTIC ACID BACTERIUM. Applicant: BENED BIOMEDICAL CO., LTD. BENED BIOMEDICAL CHINA CO., LTD. The sequence listing filed with the application follows.

SEQUENCE LISTING (5 sequences)

SEQ ID NO: 1 - DNA, 20 bp, artificial sequence
  primers for PCR amplification of 16S rDNA
agagtttgatcmtggctcag

SEQ ID NO: 2 - DNA, 20 bp, artificial sequence
  primers for PCR amplification of 16S rDNA
aaggaggtgatccaaccgca

SEQ ID NO: 3 - DNA, 1476 bp, Lactobacillus plantarum subsp. plantarum PS128
ctcaggacgaacgctggcggcgtgcctaatacatgcaagtcgaacgaactctggtattgattggtgcttgcatcatgatttacatttgagtgagtggcgaactggtgagtaacacgtgggaaacctgcccagaagcgggggataacacctggaaacagatgctaataccgcataacaacttggaccgcatggtccgagyttgaaagatggcttcggctatcacttttggatggtcccgcggcgtattagctagatggtggggtaacggctcaccatggcaatgatacgtagccgacctgagagggtaatcggccacattgggactgagacacggcccaaactcctacgggaggcagcagtagggaatcttccacaatggacgaaagtctgatggagcaacgccgcgtgagtgaagaagggtttcggctcgtaaaactctgttgttaaagaagaacatatctgagagtaactgttcaggtattgacggtatttaaccagaaagccacggctaactacgtgccagcagccgcggtaatacgtaggtggcaagcgttgtccggatttattgggcgtaaagcgagcgcaggcggttttttaagtctgatgtgaaagccttcggctcaaccgaagaagtgcatcggaaactgggaaacttgagtgcagaagaggacagtggaactccatgtgtagcggtgaaatgcgtagatatatggaagaacaccagtggcgaaggcggctgtctggtctgtaactgacgctgaggctcgaaagtatgggtagcaaacaggattagataccctggtagtccataccgtaaacgatgaatgctaagtgttggagggtttccgcccttcagtgctgcagctaacgcattaagcattccgcctggggagtacggccgcaaggctgaaactcaaaggaattgacgggggcccgcacaagcggtggagcatgtggtttaattcgaagctacgcgaagaaccttaccaggtcttgacatactatgcaaatctaagagattagacgttcccttcggggacatggatacaggtggtgcatggttgtcgtcagctcgtgtcgtgagatgttgggttaagtcccgcaacgagcgcaacccttattatcagttgccagcattaagttgggcactctggtgagactgccggtgacaaaccggaggaaggtggggatgacgtcaaatcatcatgccccttatgacctgggctacacacgtgctacaatggatggtacaacgagttgcgaactcgcgagagtaagctaatctcttaaagccattctcagttcggattgtaggctgcaactcgcctacatgaagtcggaatcgctagtaatcgcggatcagcatgccgcggtgaatacgttcccgggccttgtacacaccgcccgtcacaccatgagagtttgtaacacccaaagtcggtggggtaaccttttaggaaccagccgcctaaggtg

SEQ ID NO: 4 - DNA, 22 bp, artificial sequence
  primers for ERIC-PCR
atgtaagctcctggggattcac

SEQ ID NO: 5 - DNA, 22 bp, artificial sequence
  primers for ERIC-PCR
aagtaagtgactggggtgagcg